European Patent Application EP 4 674 407 A1, published January 7, 2026. Title: TRANSDERMAL COMPOSITION AND USE THEREOF. Applicant: KANGMA-HEATHCODE (SHANGHAI) BIOTECH CO., LTD. The sequence listing filed with the application follows.

SEQUENCE LISTING (14 sequences)

SEQ ID NO: 1 - protein, 441 aa, synthetic construct
MPFVNKQFNYKDPVNGVDIAYIKIPNVGQMQPVKAFKIHNKIWVIPERDTFTNPEEGDLNPPPEAKQVPVSYYDSTYLSTDNEKDNYLKGVTKLFERIYSTDLGRMLLTSIVRGIPFWGGSTIDTELKVIDTNCINVIQPDGSYRSEELNLVIIGPSADIIQFECKSFGHEVLNLTRNGYGSTQYIRFSPDFTFGFEESLEVDTNPLLGAGKFATDPAVTLAHELIHAGHRLYGIAINPNRVFKVNTNAYYEMSGLEVSFEELRTFGGHDAKFIDSLQENEFRLYYYNKFKDIASTLNKAKSIVGTTASLQYMKNVFKEKYLLSEDTSGKFSVDKLKFDKLYKMLTEIYTEDNFVKFFKVLNRKTYLNFDKAVFKINIVPKVNYTIYDGFNLRNTNLAANFNGQNTEINNMNFTKLKNFTGLFEFYKLLCVRGIITSQTQS

SEQ ID NO: 2 - protein, 441 aa, synthetic construct
MPVTINNFNYNDPIDNNNIIMMEPPFARGTGRYYKAFKITDRIWIIPERYTFGYKPEDFNKSSGIFNRDVCEYYDPDYLNTNDKKNIFLQTMIKLFNRIKSKPLGEKLLEMIINGIPYLGDRRVPLEEFNTNIASVTVNKLISNPGEVERKKGIFANLIIFGPGPVLNENETIDIGIQNHFASREGFGGIMQMKFCPEYVSVFNNVQENKGASIFNRRGYFSDPALILMHELIHVLHGLYGIKVDDLPIVPNEKKFFMQSTDAIQAEELYTFGGQDPSIITPSTDKSIYDKVLQNFRGIVDRLNKVLVCISDPNININIYKNKFKDKYKFVEDSEGKYSIDVESFDKLYKSLMFGFTETNIAENYKIKTRASYFSDSLPPVKIKNLLDNEIYTIEEGFNISDKNMEKEYRGQNKAINKQAYEEISKEHLAVYKIQMCKSVR

SEQ ID NO: 3 - protein, 444 aa, synthetic construct
MPITINNFNYSDPVDNKNILYLDTHLNTLANEPEKAFRITGNIWVIPDRFSRNSNPNLNKPPRVTSPKSGYYDPNYLSTDSDKDTFLKEIIKLFKRINSREIGEELIYRLSTDIPFPGNNNTPINTFDFDVDFNSVDVKTRQGNNWVKTGSINPSVIITGPRENIIDPETSTFKLTNNTFAAQEGFGALSIISISPRFMLTYSNATNDVGEGRFSKSEFCMDPILILMHELNHAMHNLYGIAIPNDQTISSVTSNIFYSQYNVKLEYAEIYAFGGPTIDLIPKSARKYFEEKALDYYRSIAKRLNSITTANPSSFNKYIGEYKQKLIRKYRFVVESSGEVTVNRNKFVELYNELTQIFTEFNYAKIYNVQNRKIYLSNVYTPVTANILDDNVYDIQNGFNIPKSNLNVLFMGQNLSRNPALRKVNPENMLYLFTKFCHKAIDGR

SEQ ID NO: 4 - protein, 445 aa, synthetic construct
MTWPVKDFNYSDPVNDNDILYLRIPQNKLITTPVKAFMITQNIWVIPERFSSDTNPSLSKPPRPTSKYQSYYDPSYLSTDEQKDTFLKGIIKLFKRINERDIGKKLINYLVVGSPFMGDSSTPEDTFDFTRHTTNIAVEKFENGSWKVTNIITPSVLIFGPLPNILDYTASLTLQGQQSNPSFEGFGTLSILKVAPEFLLTFSDVTSNQSSAVLGKSIFCMDPVIALMHELTHSLHQLYGINIPSDKRIRPQVSEGFFSQDGPNVQFEELYTFGGLDVEIIPQIERSQLREKALGHYKDIAKRLNNINKTIPSSWISNIDKYKKIFSEKYNFDKDNTGNFVVNIDKFNSLYSDLTNVMSEVVYSSQYNVKNRTHYFSRHYLPVFANILDDNIYTIRDGFNLTNKGFNIENSGQNIERNPALQKLSSESVVDLFTKVCLRLTKNSR

SEQ ID NO: 5 - protein, 422 aa, synthetic construct
MPTINSFNYNDPVNNRTILYIKPGGCQQFYKSFNIMKNIWIIPERNVIGTIPQDFLPPTSLKNGDSSYYDPNYLQSDQEKDKFLKIVTKIFNRINDNLSGRILLEELSKANPYLGNDNTPDGDFIINDASAVPIQFSNGSQSILLPNVIIMGAEPDLFETNSSNISLRNNYMPSNHGFGSIAIVTFSPEYSFRFKDNSMNEFIQDPALTLMHELIHSLHGLYGAKGITTKYTITQKQNPLITNIRGTNIEEFLTFGGTDLNIITSAQSNDIYTNLLADYKKIASKLSKVQVSNPLLNPYKDVFEAKYGLDKDASGIYSVNINKFNDIFKKLYSFTEFDLATKFQVKCRQTYIGQYKYFKLSNLLNDSIYNISEGYNINNLKVNFRGQNANLNPRIITPITGRGLVKKIIRFCKNIVSVKGIR

SEQ ID NO: 6 - protein, 439 aa, synthetic construct
MPVAINSFNYNDPVNDDTILYMQIPYEEKSKKYYKAFEIMRNVWIIPERNTIGTNPSDFDPPASLKNGSSAYYDPNYLTTDAEKDRYLKTTIKLFKRINSNPAGKVLLQEISYAKPYLGNDHTPIDEFSPVTRTTSVNIKLSTNVESSMLLNLLVLGAGPDIFESCCYPVRKLIDPDVVYDPSNYGFGSINIVTFSPEYEYTFNDISGGHNSSTESFIADPAISLAHELIHALHGLYGARGVTYEETIEVKQAPLMIAEKPIRLEEFLTFGGQDLNIITSAMKEKIYNNLLANYEKIATRLSEVNSAPPEYDINEYKDYFQWKYGLDKNADGSYTVNENKFNEIYKKLYSFTESDLANKFKVKCRNTYFIKYEFLKVPNLLDDDIYTVSEGFNIGNLAVNNRGQSIKLNPKIIDSIPDKGLVEKIVKFCKSVIPRKGTK

SEQ ID NO: 7 - protein, 446 aa, synthetic construct
MPVNIKXFNYNDPINNDDIIMMEPFNDPGPGTYYKAFRIIDRIWIVPERFTYGFQPDQFNASTGVFSKDVYEYYDPTYLKTDAEKDKFLKTMIKLFNRINSKPSGQRLLDMIVDAIPYLGNASTPPDKFAANVANVSINKKIIQPGAEDQIKGLMTNLIIFGPGPVLSDNFTDSMIMNGHSPISEGFGARMMIRFCPSCLNVFNNVQENKDTSIFSRRAYFADPALTLMHELIHVLHGLYGIKISNLPITPNTKEFFMQHSDPVQAEELYTFGGHDPSVISPSTDMNIYNKALQNFQDIANRLNIVSSAQGSGIDISLYKQIYKNKYDFVEDPNGKYSVDKDKFDKLYKALMFGFTETNLAGEYGIKTRYSYFSEYLPPIKTEKLLDNTIYTQNEGFNIASKNLKTEFNGQNKAVNKEAYEEISLEHLVIYRIAMCKPVMYKNTGK

SEQ ID NO: 8 - protein, 848 aa, synthetic construct
ALNDLCIKVNNWDLFFSPSEDNFTNDLNKGEEITSDTNIEAAEENISLDLIQQYYLTFNFDNEPENISIENLSSDIIGQLELMPNIERFPNGKKYELDKYTMFHYLRAQEFEHGKSRIALTNSVNEALLNPSRVYTFFSSDYVKKVNKATEAAMFLGWVEQLVYDFTDETSEVSTTDKIADITIIIPYIGPALNIGNMLYKDDFVGALIFSGAVILLEFIPEIAIPVLGTFALVSYIANKVLTVQTIDNALSKRNEKWDEVYKYIVTNWLAKVNTQIDLIRKKMKEALENQAEATKAIINYQYNQYTEEEKNNINFNIDDLSSKLNESINKAMININKFLNQCSVSYLMNSMIPYGVKRLEDFDASLKDALLKYIYDNRGTLIGQVDRLKDKVNNTLSTDIPFQLSKYVDNQRLLSTFTEYINNIINTSILNLRYESNHLIDLSRYASKINIGSKVNFDPIDKNQIQLFNLESSKIEVILKNAIVYNSMYENFSTSFWIRIPKYFNSISLNNEYTIINCMENNSGWKVSLNYGEIIWTLQDTQEIKQRVVFKYSQMINISDYINRWIFVTITNNRLNNSKIYINGRLIDQKPISNLGNIHASNNIMFKLDGCRDTHRYIWIKYFNLFDKELNEKEIKDLYDNQSNSGILKDFWGDYLQYDKPYYMLNLYDPNKYVDVNNVGIRGYMYLKGPRGSVMTTNIYLNSSLYRGTKFIIKKYASGNKDNIVRNNDRVYINVVVKNKEYRLATNASQAGVEKILSALEIPDVGNLSQVVVMKSKNDQGITNKCKMNLQDNNGNDIGFIGFHQFNNIAKLVASNWYNRQIERSSRTLGCSWEFIPVDDGWGERPL

SEQ ID NO: 9 - protein, 850 aa, synthetic construct
APGICIDVDNEDLFFIADKNSFSDDLSKNERIEYDTQSNYIENRSSINELILDTNLISKIELPSENTESLTDFNVDVPVYEKQPAIKKIFTDENTIFQYLYSQTFPLDIRDISLTSSFDDALLFSNKVYSFFSMDYIKTANKVVEAGLFAGWVKQIVDDFVIEANKSSTMDKIADISLIVPYIGLALNVGNETAKGNFENAFEIAGASILLEFIPELLIPVVGAFLLESYIDNKNKIIKTIDNALTKRDEKWIDMYGLIVAQWLSTVNTQFYTIKEGMYKALNYQAQALEEIIKYKYNIYSEKEKSNINIDFNDINSKLNEGINQAIDNINDFINECSVSYLMKKMIPLAVEKLLDFDNTLKKNLLNYIDENKLYLIGSAEYEKSKVDKYLKTIIPFDLSMYTNNTILIEIFNKYNSEILNNIILNLRYRDNNLIDLSGYGANVEVYDGVKLNDKNQFKLTSSTNSEIRVTQNQNIIFNSMFLDFSVSFWIRIPKYKNDGIQNYIHNEYTIINCIKNNSGWKISIRGNRIIWTLTDINGKTKSVFFEYSIREDISDYINRWFFVTITNNSDNAKIYINGKLESNIDIKNIGEVIANGEIIFKLDGDIDRTQFIWMKYFSIFNTELSQSNIKEIYKIQSYSEYLKDFWGNPLMYNKEYYMFNAGNKNSYIKLKKDSSVGEILTRSKYNQNSNYINYRNLYIGEKFIIRRKSNSQSINDDIVRKEDYIYLDFFNSNREWRVYAYKDFKEEEKKLFLANIYDSNEFYKTIQIKEYDEQPTYSCQLLFKKDEESTDEIGLIGIHRFYESGIVLKDYKNYFCISKWYLKEVKRKPYNPNLGCNWQFIPKDEGWIE

SEQ ID NO: 10 - protein, 847 aa, synthetic construct
SLYNKTLDCRELLVKNTDLPFIGDISDVKTDIFLRKDINEETEVIYYPDNVSVDQVILSKNTSEHGQLDLLYPSIDSESEILPGENQVFYDNRTQNVDYLNSYYYLESQKLSDNVEDFTFTRSIEEALDNSAKVYTYFPTLANKVNAGVQGGLFLMWANDVVEDFTTNILRKDTLDKISDVSAIIPYIGPALNISNSVRRGNFTEAFAVTGVTILLEAFPEFTIPALGAFVIYSKVQERNEIIKTIDNCLEQRIKRWKDSYEWMMGTWLSRIITQFNNISYQMYDSLNYQAGAIKAKIDLEYKKYSGSDKENIKSQVENLKNSLDVKISEAMNNINKFIRECSVTYLFKNMLPKVIDELNEFDRNTKAKLINLIDSHNIILVGEVDKLKAKVNNSFQNTIPFNIFSYTNNSLLKDIINEYFNNINDSKILSLQNRKNTLVDTSGYNAEVSEEGDVQLNPIFPFDFKLGSSGEDRGKVIVTQNENIVYNSMYESFSISFWIRINKWVSNLPGYTIIDSVKNNSGWSIGIISNFLVFTLKQNEDSEQSINFSYDISNNAPGYNKWFFVTVTNNMMGNMKIYINGKLIDTIKVKELTGINFSKTITFEINKIPDTGLITSDSDNINMWIRDFYIFAKELDGKDINILFNSLQYTNVVKDYWGNDLRYNKEYYMVNIDYLNRYMYANSRQIVFNTRRNNNDFNEGYKIIIKRIRGNTNDTRVRGGDILYFDMTINNKAYNLFMKNETMYADNHSTEDIYAIGLREQTKDINDNIIFQIQPMNNTYYYASQIFKSNFNGENISGICSIGTYRFRLGGDWYRHNYLVPTVKQGNYASLLESTSTHWGFVPVSE

SEQ ID NO: 11 - protein, 831 aa, synthetic construct
DDSTCIKVKNNRLPYVADKDSISQEIFENKIITDETNVQNYSDKFSLDESILDGQVPINPEIVDPLLPNVNMEPLNLPGEEIVFYDDITKYVDYLNSYYYLESQKLSNNVENITLTTSVEEALGYSNKIYTFLPSLAEKVNKGVQAGLFLNWANEVVEDFTTNIMKKDTLDKISDVSVIIPYIGPALNIGNSALRGNFNQAFATAGVAFLLEGFPEFTIPALGVFTFYSSIQEREKIIKTIENCLEQRVKRWKDSYQWMVSNWLSRITTQFNHINYQMYDSLSYQADAIKAKIDLEYKKYSGSDKENIKSQVENLKNSLDVKISEAMNNINKFIRECSVTYLFKNMLPKVIDELNKFDLRTKTELINLIDSHNIILVGEVDRLKAKVNESFENTMPFNIFSYTNNSLLKDIINEYFNSINDSKILSLQNKKNALVDTSGYNAEVRVGDNVQLNTIYTNDFKLSSSGDKIIVNLNNNILYSAIYENSSVSFWIKISKDLTNSHNEYTIINSIEQNSGWKLCIRNGNIEWILQDVNRKYKSLIFDYSESLSHTGYTNKWFFVTITNNIMGYMKLYINGELKQSQKIEDLDEVKLDKTIVFGIDENIDENQMLWIRDFNIFSKELSNEDINIVYEGQILRNVIKDYWGNPLKFDTEYYIINDNYIDRYIAPESNVLVLVQYPDRSKLYTGNPITIKSVSDKNPYSRILNGDNIILHMLYNSRKYMIIRDTDTIYATQGGECSQNCVYALKLQSNLGNYGIGIFSIKNIVSKNKYCSQIFSSFRENTMLLADIYKPWRFSFKNAYTPVAVTNYETKLLSTSSFWKFISRDPGWVE

SEQ ID NO: 12 - protein, 829 aa, synthetic construct
KSICIEINNGELFFVASENSYNDDNINTPKEIDDTVTSNNNYENDLDQVILNFNSESAPGLSDEKLNLTIQNDAYIPKYDSNGTSDIEQHDVNELNVFFYLDAQKVPEGENNVNLTSSIDTALLEQPKIYTFFSSEFINNVNKPVQAALFVGWIQQVLVDFTTEANQKSTVDKIADISIVVPYIGLALNIGNEAQKGNFKDALELLGAGILLEFEPELLIPTILVFTIKSFLGSSDNKNKVIKAINNALKERDEKWKEVYSFIVSNWMTKINTQFNKRKEQMYQALQNQVNALKAIIESKYNSYTLEEKNELTNKYDIEQIENELNQKVSIAMNNIDRFLTESSISYLMKLINEVKINKLREYDENVKTYLLDYIIKHGSILGESQQELNSMVIDTLNNSIPFKLSSYTDDKILISYFNKFFKRIKSSSVLNMRYKNDKYVDTSGYDSNININGDVYKYPTNKNQFGIYNDKLSEVNISQNDYIIYDNKYKNFSISFWVRIPNYDNKIVNVNNEYTIINCMRDNNSGWKVSLNHNEIIWTLQDNSGINQKLAFNYGNANGISDYINKWIFVTITNDRLGDSKLYINGNLIDKKSILNLGNIHVSDNILFKIVNCSYTRYIGIRYFNIFDKELDETEIQTLYNNEPNANILKDFWGNYLLYDKEYYLLNVLKPNNFINRRTDSTLSINNIRSTILLANRLYSGIKVKIQRVNNSSTNDNLVRKNDQVYINFVASKTHLLPLYADTATTNKEKTIKISSSGNRFNQVVVMNSVGNCTMNFKNNNGNNIGLLGFKADTVVASTWYYTHMRDNTNSNGFFWNFISEEHGWQEK

SEQ ID NO: 13 - protein, 835 aa, synthetic construct
APPRLCIRVNNSELFFVASESSYNENDINTPKEIDDTTNLNNNYRNNLDEVILDYNSQTIPQISNRTLNTLVQDNSYVPRYDSNGTSEIEEYDVVDFNVFFYLHAQKVPEGETNISLTSSIDTALLEESKDIFFSSEFIDTINKPVNAALFIDWISKVIRDFTTEATQKSTVDKIADISLIVPYVGLALNIIIEAEKGNFEEAFELLGVGILLEFVPELTIPVILVFTIKSYIDSYENKNKAIKAINNSLIEREAKWKEIYSWIVSNWLTRINTQFNKRKEQMYQALQNQVDAIKTAIEYKYNNYTSDEKNRLESEYNINNIEEELNKKVSLAMKNIERFMTESSISYLMKLINEAKVGKLKKYDNHVKSDLLNYILDHRSILGEQTNELSDLVTSTLNSSIPFELSSYTNDKILIIYFNRLYKKIKDSSILDMRYENNKFIDISGYGSNISINGNVYIYSTNRNQFGIYNSRLSEVNIAQNNDIIYNSRYQNFSISFWVRIPKHYKPMNHNREYTIINCMGNNNSGWKISLRTVRDCEIIWTLQDTSGNKENLIFRYEELNRISNYINKWIFVTITNNRLGNSRIYINGNLIVEKSISNLGDIHVSDNILFKIVGCDDETYVGIRYFKVFNTELDKTEIETLYSNEPDPSILKNYWGNYLLYNKKYYLFNLLRKDKYITLNSGILNINQQRGVTEGSVFLNYKLYEGVEVIIRKNGPIDISNTDNFVRKNDLAYINVVDRGVEYRLYADTKSEKEKIIRTSNLNDSLGQIIVMDSIGNNCTMNFQNNNGSNIGLLGFHSNNLVASSWYYNNIRRNTSSNGCFWSSISKENGWKE

SEQ ID NO: 14 - protein, 851 aa, synthetic construct
SEQCIIVNNEDLFFIANKDSFSKDLAKAETIAYNTQNNTIENNFSIDQLILDNDLSSGIDLPNENTEPFTNFDDIDIPVYIKQSALKKIFVDGDSLFEYLHAQTFPSNIENLQLTNSLNDALRNNNKVYTFFSTNLVEKANTVVGASLFVNWVKGVIDDFTSESTQKSTIDKVSDVSIIIPYIGPALNVGNETAKENFKNAFEIGGAAILMEFIPELIVPIVGFFTLESYVGNKGHIIMTISNALKKRDQKWTDMYGLIVSQWLSTVNTQFYTIKERMYNALNNQSQAIEKIIEDQYNRYSEEDKMNINIDFNDIDFKLNQSINLAINNIDDFINQCSISYLMNRMIPLAVKKLKDFDDNLKRDLLEYIDTNELYLLDEVNILKSKVNRHLKDSIPFDLSLYTKDTILIQVFNNYISNISSNAILSLSYRGGRLIDSSGYGATMNVGSDVIFNDIGNGQFKLNNSENSNITAHQSKFVVYDSMFDNFSINFWVRTPKYNNNDIQTYLQNEYTIISCIKNDSGWKVSIKGNRIIWTLIDVNAKSKSIFFEYSIKDNISDYINKWFSITITNDRLGNANIYINGSLKKSEKILNLDRINSSNDIDFKLINCTDTTKFVWIKDFNIFGRELNATEVSSLYWIQSSTNTLKDFWGNPLRYDTQYYLFNQGMQNIYIKYFSKASMGETAPRTNFNNAAINYQNLYLGLRFIIKKASNSRNINNDNIVREGDYIYLNIDNISDESYRVYVLVNSKEIQTQLFLAPINDDPTFYDVLQIKKYYEKTTYNCQILCEKDTKTFGLFGIGKFVKDYGYVWDTYDNYFCISQWYLRRISENINKLRLGCNWQFIPVDEGWTE